European Patent Application EP 4 219 730 A1, published August 2, 2023. Title: Method For Conducting Site-Specific Modification on Entire Plant Via Gene Transient Expression. Applicant: Institute of Genetics and Developmental Biology, Chinese. The sequence listing filed with the application follows.

SEQUENCE LISTING (51 sequences)

SEQ ID NO: 1 - DNA, 883 bp, synthetic construct
  misc_feature 1..883: note = pZmU3-gRNA-C1
  source 1..883: mol_type = other DNA
gaattccatctaagtatcttggtaaagcatggattaatttggatgcccacttcaggtctatgcagctccggtgccttgtgattgtgagttgtgaccgatgctcatgctattctgcatttctgcgatgtatgtagctagtagatcttcaaaactaacaccgcatgccatcatcatccactgcttgattttagtctcaccgctggccaaaaatgtgatgatgccagaaacctcaactaccttgaatcaacacgggcccaacagtgtgatgacgacagaaacaaaaaaaaatgagccaatagttcagaaggaggcactatgcagaaactacatttctgaaggtgactaaaaggtgagcgtagagtgtaattactagtagtttagccaccattacccaaatgctttcgagcttgtattaagatttcctaagctgagcatcatcactgatctgcaggccaccctcgcttcgctgccaagatcaacagcaaccatgtggcggcaacatccagcattgcacatgggctaaagattgagctttgtgcctcgtctagggatcagctgaggttatcagtctttcctttttttcatccaggtgaggcatcaagctactactgcctcgattggctggacccgaagcccacatgtaggataccagaatgggccgacccaggacgcagtatgttggccagtcccaccggttagtgccatctcggttgctcacatgcgtagaagccagcttaaaaatttagctttggtgactcacagcagtcggcggcgtggtcgagctgttttagagctagaaatagcaagttaaaataaggctagtccgttatcaacttgaaaaagtggcaccgagtcggtgctttttttggtaccggatcctacg

SEQ ID NO: 2 - DNA, 4206 bp, synthetic construct
  misc_feature 1..4206: note = Cas9 sequence in pJIT163-Ubi-Cas9
  source 1..4206: mol_type = other DNA
atggcccctaagaagaagagaaaggtcggtattcacggcgttcctgcggcgatggacaagaagtatagtattggtctggacattgggacgaattccgttggctgggccgtgatcaccgatgagtacaaggtcccttccaagaagtttaaggttctggggaacaccgatcggcacagcatcaagaagaatctcattggagccctcctgttcgactcaggcgagaccgccgaagcaacaaggctcaagagaaccgcaaggagacggtatacaagaaggaagaataggatctgctacctgcaggagattttcagcaacgaaatggcgaaggtggacgattcgttctttcatagattggaggagagtttcctcgtcgaggaagataagaagcacgagaggcatcctatctttggcaacattgtcgacgaggttgcctatcacgaaaagtaccccacaatctatcatctgcggaagaagcttgtggactcgactgataaggcggaccttagattgatctacctcgctctggcacacatgattaagttcaggggccattttctgatcgagggggatcttaacccggacaatagcgatgtggacaagttgttcatccagctcgtccaaacctacaatcagctctttgaggaaaacccaattaatgcttcaggcgtcgacgccaaggcgatcctgtctgcacgcctttcaaagtctcgccggcttgagaacttgatcgctcaactcccgggcgaaaagaagaacggcttgttcgggaatctcattgcactttcgttggggctcacaccaaacttcaagagtaattttgatctcgctgaggacgcaaagctgcagctttccaaggacacttatgacgatgacctggataaccttttggcccaaatcggcgatcagtacgcggacttgttcctcgccgcgaagaatttgtcggacgcgatcctcctgagtgatattctccgcgtgaacaccgagattacaaaggccccgctctcggcgagtatgatcaagcgctatgacgagcaccatcaggatctgacccttttgaaggctttggtccggcagcaactcccagagaagtacaaggaaatcttctttgatcaatccaagaacggctacgctggttatattgacggcggggcatcgcaggaggaattctacaagtttatcaagccaattctggagaagatggatggcacagaggaactcctggtgaagctcaatagggaggaccttttgcggaagcaaagaactttcgataacggcagcatccctcaccagattcatctcggggagctgcacgccatcctgagaaggcaggaagacttctacccctttcttaaggataaccgggagaagatcgaaaagattctgacgttcagaattccgtactatgtcggaccactcgcccggggtaattccagatttgcgtggatgaccagaaagagcgaggaaaccatcacaccttggaacttcgaggaagtggtcgataagggcgcttccgcacagagcttcattgagcgcatgacaaattttgacaagaacctgcctaatgagaaggtccttcccaagcattccctcctgtacgagtatttcactgtttataacgaactcacgaaggtgaagtatgtgaccgagggaatgcgcaagcccgccttcctgagcggcgagcaaaagaaggcgatcgtggaccttttgtttaagaccaatcggaaggtcacagttaagcagctcaaggaggactacttcaagaagattgaatgcttcgattccgttgagatcagcggcgtggaagacaggtttaacgcgtcactggggacttaccacgatctcctgaagatcattaaggataaggacttcttggacaacgaggaaaatgaggatatcctcgaagacattgtcctgactcttacgttgtttgaggatagggaaatgatcgaggaacgcttgaagacgtatgcccatctcttcgatgacaaggttatgaagcagctcaagagaagaagatacaccggatggggaaggctgtcccgcaagcttatcaatggcattagagacaagcaatcagggaagacaatccttgactttttgaagtctgatggcttcgcgaacaggaattttatgcagctgattcacgatgactcacttactttcaaggaggatatccagaaggctcaagtgtcgggacaaggtgacagtctgcacgagcatatcgccaaccttgcgggatctcctgcaatcaagaagggtattctgcagacagtcaaggttgtggatgagcttgtgaaggtcatgggacggcataagcccgagaacatcgttattgagatggccagagaaaatcagaccacacaaaagggtcagaagaactcgagggagcgcatgaagcgcatcgaggaaggcattaaggagctggggagtcagatccttaaggagcacccggtggaaaacacgcagttgcaaaatgagaagctctatctgtactatctgcaaaatggcagggatatgtatgtggaccaggagttggatattaaccgcctctcggattacgacgtcgatcatatcgttcctcagtccttccttaaggatgacagcattgacaataaggttctcaccaggtccgacaagaaccgcgggaagtccgataatgtgcccagcgaggaagtcgttaagaagatgaagaactactggaggcaacttttgaatgccaagttgatcacacagaggaagtttgataacctcactaaggccgagcgcggaggtctcagcgaactggacaaggcgggcttcattaagcggcaactggttgagactagacagatcacgaagcacgtggcgcagattctcgattcacgcatgaacacgaagtacgatgagaatgacaagctgatccgggaagtgaaggtcatcaccttgaagtcaaagctcgtttctgacttcaggaaggatttccaattttataaggtgcgcgagatcaacaattatcaccatgctcatgacgcatacctcaacgctgtggtcggaacagcattgattaagaagtacccgaagctcgagtccgaattcgtgtacggtgactataaggtttacgatgtgcgcaagatgatcgccaagtcagagcaggaaattggcaaggccactgcgaagtatttcttttactctaacattatgaatttctttaagactgagatcacgctggctaatggcgaaatccggaagagaccacttattgagaccaacggcgagacaggggaaatcgtgtgggacaaggggagggatttcgccacagtccgcaaggttctctctatgcctcaagtgaatattgtcaagaagactgaagtccagacgggcgggttctcaaaggaatctattctgcccaagcggaactcggataagcttatcgccagaaagaaggactgggacccgaagaagtatggaggtttcgactcaccaacggtggcttactctgtcctggttgtggcaaaggtggagaagggaaagtcaaagaagctcaagtctgtcaaggagctcctgggtatcaccattatggagaggtccagcttcgaaaagaatccgatcgattttctcgaggcgaagggatataaggaagtgaagaaggacctgatcattaagcttccaaagtacagtcttttcgagttggaaaacggcaggaagcgcatgttggcttccgcaggagagctccagaagggtaacgagcttgctttgccgtccaagtatgtgaacttcctctatctggcatcccactacgagaagctcaagggcagcccagaggataacgaacagaagcaactgtttgtggagcaacacaagcattatcttgacgagatcattgaacagatttcggagttcagtaagcgcgtcatcctcgccgacgcgaatttggataaggttctctcagcctacaacaagcaccgggacaagcctatcagagagcaggcggaaaatatcattcatctcttcaccctgacaaaccttggggctcccgctgcattcaagtattttgacactacgattgatcggaagagatacacttctacgaaggaggtgctggatgcaacccttatccaccaatcgattactggcctctacgagacgcggatcgacttgagtcagctcgggggggataagagaccagcggcaaccaagaaggcaggacaagcgaagaagaagaagtag

SEQ ID NO: 3 - DNA, 544 bp, synthetic construct
  misc_feature 1..544: note = gRNA sequence of pBUE411-C1
  source 1..544: mol_type = other DNA
agtaattcatccaggtctccaagttctaggattttcagaactgcaacttattttatcaaggaatctttaaacatacgaacagatcacttaaagttcttctgaagcaacttaaagttatcaggcatgcatggatcttggaggaatcagatgtgcagtcagggaccatagcacaagacaggcgtcttctactggtgctaccagcaaatgctggaagccgggaacactgggtacgttggaaaccacgtgatgtgaagaagtaagataaactgtaggagaaaagcatttcgtagtgggccatgaagcctttcaggacatgtattgcagtatgggccggcccattacgcaattggacgacaacaaagactagtattagtaccacctcggctatccacatagatcaaagctgatttaaaagagttgtgcagatgatccgtggcggtcggcggcgtggtcgagctgttttagagctagaaatagcaagttaaaataaggctagtccgttatcaacttgaaaaagtggcaccgagtcggtgctttttttttt

SEQ ID NO: 4 - DNA, 4272 bp, synthetic construct
  misc_feature 1..4272: note = Cas9 sequence of pHSN411-C1
  source 1..4272: mol_type = other DNA
atggattacaaggaccacgacggggattacaaggaccacgacattgattacaaggatgatgatgacaagatggctccgaagaagaagaggaaggttggcatccacggggtgccagctgctgacaagaagtactcgatcggcctcgatattgggactaactctgttggctgggccgtgatcaccgacgagtacaaggtgccctcaaagaagttcaaggtcctgggcaacaccgatcggcattccatcaagaagaatctcattggcgctctcctgttcgacagcggcgagacggctgaggctacgcggctcaagcgcaccgcccgcaggcggtacacgcgcaggaagaatcgcatctgctacctgcaggagattttctccaacgagatggcgaaggttgacgattctttcttccacaggctggaggagtcattcctcgtggaggaggataagaagcacgagcggcatccaatcttcggcaacattgtcgacgaggttgcctaccacgagaagtaccctacgatctaccatctgcggaagaagctcgtggactccacagataaggcggacctccgcctgatctacctcgctctggcccacatgattaagttcaggggccatttcctgatcgagggggatctcaacccggacaatagcgatgttgacaagctgttcatccagctcgtgcagacgtacaaccagctcttcgaggagaaccccattaatgcgtcaggcgtcgacgcgaaggctatcctgtccgctaggctctcgaagtctcggcgcctcgagaacctgatcgcccagctgccgggcgagaagaagaacggcctgttcgggaatctcattgcgctcagcctggggctcacgcccaacttcaagtcgaatttcgatctcgctgaggacgccaagctgcagctctccaaggacacatacgacgatgacctggataacctcctggcccagatcggcgatcagtacgcggacctgttcctcgctgccaagaatctgtcggacgccatcctcctgtctgatattctcagggtgaacaccgagattacgaaggctccgctctcagcctccatgatcaagcgctacgacgagcaccatcaggatctgaccctcctgaaggcgctggtcaggcagcagctccccgagaagtacaaggagatcttcttcgatcagtcgaagaacggctacgctgggtacattgacggcggggcctctcaggaggagttctacaagttcatcaagccgattctggagaagatggacggcacggaggagctgctggtgaagctcaatcgcgaggacctcctgaggaagcagcggacattcgataacggcagcatcccacaccagattcatctcggggagctgcacgctatcctgaggaggcaggaggacttctaccctttcctcaaggataaccgcgagaagatcgagaagattctgactttcaggatcccgtactacgtcggcccactcgctaggggcaactcccgcttcgcttggatgacccgcaagtcagaggagacgatcacgccgtggaacttcgaggaggtggtcgacaagggcgctagcgctcagtcgttcatcgagaggatgacgaatttcgacaagaacctgccaaatgagaaggtgctccctaagcactcgctcctgtacgagtacttcacagtctacaacgagctgactaaggtgaagtatgtgaccgagggcatgaggaagccggctttcctgtctggggagcagaagaaggccatcgtggacctcctgttcaagaccaaccggaaggtcacggttaagcagctcaaggaggactacttcaagaagattgagtgcttcgattcggtcgagatctctggcgttgaggaccgcttcaacgcctccctggggacctaccacgatctcctgaagatcattaaggataaggacttcctggacaacgaggagaatgaggatatcctcgaggacattgtgctgacactcactctgttcgaggaccgggagatgatcgaggagcgcctgaagacttacgcccatctcttcgatgacaaggtcatgaagcagctcaagaggaggaggtacaccggctgggggaggctgagcaggaagctcatcaacggcattcgggacaagcagtccgggaagacgatcctcgacttcctgaagagcgatggcttcgcgaaccgcaatttcatgcagctgattcacgatgacagcctcacattcaaggaggatatccagaaggctcaggtgagcggccagggggactcgctgcacgagcatatcgcgaacctcgctggctcgccagctatcaagaaggggattctgcagaccgtgaaggttgtggacgagctggtgaaggtcatgggcaggcacaagcctgagaacatcgtcattgagatggcccgggagaatcagaccacgcagaagggccagaagaactcacgcgagaggatgaagaggatcgaggagggcattaaggagctggggtcccagatcctcaaggagcacccggtggagaacacgcagctgcagaatgagaagctctacctgtactacctccagaatggccgcgatatgtatgtggaccaggagctggatattaacaggctcagcgattacgacgtcgatcatatcgttccacagtcattcctgaaggatgactccattgacaacaaggtcctcaccaggtcggacaagaaccggggcaagtctgataatgttccttcagaggaggtcgttaagaagatgaagaactactggcgccagctcctgaatgccaagctgatcacgcagcggaagttcgataacctcacaaaggctgagaggggcgggctctctgagctggacaaggcgggcttcatcaagaggcagctggtcgagacacggcagatcactaagcacgttgcgcagattctcgactcacggatgaacactaagtacgatgagaatgacaagctgatccgcgaggtgaaggtcatcaccctgaagtcaaagctcgtctccgacttcaggaaggatttccagttctacaaggttcgggagatcaacaattaccaccatgcccatgacgcgtacctgaacgcggtggtcggcacagctctgatcaagaagtacccaaagctcgagagcgagttcgtgtacggggactacaaggtttacgatgtgaggaagatgatcgccaagtcggagcaggagattggcaaggctaccgccaagtacttcttctactctaacattatgaatttcttcaagacagagatcactctggccaatggcgagatccggaagcgccccctcatcgagacgaacggcgagacgggggagatcgtgtgggacaagggcagggatttcgcgaccgtcaggaaggttctctccatgccacaagtgaatatcgtcaagaagacagaggtccagactggcgggttctctaaggagtcaattctgcctaagcggaacagcgacaagctcatcgcccgcaagaaggactgggatccgaagaagtacggcgggttcgacagccccactgtggcctactcggtcctggttgtggcgaaggttgagaagggcaagtccaagaagctcaagagcgtgaaggagctgctggggatcacgattatggagcgctccagcttcgagaagaacccgatcgatttcctggaggcgaagggctacaaggaggtgaagaaggacctgatcattaagctccccaagtactcactcttcgagctggagaacggcaggaagcggatgctggcttccgctggcgagctgcagaaggggaacgagctggctctgccgtccaagtatgtgaacttcctctacctggcctcccactacgagaagctcaagggcagccccgaggacaacgagcagaagcagctgttcgtcgagcagcacaagcattacctcgacgagatcattgagcagatttccgagttctccaagcgcgtgatcctggccgacgcgaatctggataaggtcctctccgcgtacaacaagcaccgcgacaagccaatcagggagcaggctgagaatatcattcatctcttcaccctgacgaacctcggcgcccctgctgctttcaagtacttcgacacaactatcgatcgcaagaggtacacaagcactaaggaggtcctggacgcgaccctcatccaccagtcgattaccggcctctacgagacgcgcatcgacctgtctcagctcgggggcgacaagcggccagcggcgacgaagaaggcggggcaggcgaagaagaagaagtga

SEQ ID NO: 5 - DNA, 487 bp, synthetic construct
  misc_feature 1..487: note = partial gDNA sequence of pHSN401-C2
  source 1..487: mol_type = other DNA
aagcttcgacttgccttccgcacaatacatcatttcttcttagctttttttcttcttcttcgttcatacagtttttttttgtttatcagcttacattttcttgaaccgtagctttcgttttcttctttttaactttccattcggagtttttgtatcttgtttcatagtttgtcccaggattagaatgattaggcatcgaaccttcaagaatttgattgaataaaacatcttcattcttaagatatgaagataatcttcaaaaggcccctgggaatctgaaagaagagaagcaggcccatttatatgggaaagaacaatagtatttcttatataggcccatttaagttgaaaacaatcttcaaaagtcccacatcgcttagataagaaaacgaagctgagtttatatacagctagagtcgaagtagtgattggtgaaatcggcggatatcgtgttttagagctagaaatagcaagttaaaataaggct

SEQ ID NO: 6 - DNA, 20 bp, Zea mays
  source 1..20: mol_type = genomic DNA
agctcgaccacgccgccgac

SEQ ID NO: 7 - DNA, 24 bp, synthetic construct
  misc_feature 1..24: note = fragment inserted in pZmU3-gRNA
  source 1..24: mol_type = other DNA
agcagtcggcggcgtggtcgagct

SEQ ID NO: 8 - DNA, 24 bp, synthetic construct
  misc_feature 1..24: note = fragment inserted in pBUE411
  source 1..24: mol_type = other DNA
ggcggtcggcggcgtggtcgagct

SEQ ID NO: 9 - DNA, 20 bp, Arabidopsis thaliana
  source 1..20: mol_type = genomic DNA
acgatatccgccgatttcac

SEQ ID NO: 10 - DNA, 24 bp, synthetic construct
  misc_feature 1..24: note = fragment inserted in pHSN401
  source 1..24: mol_type = other DNA
attggtgaaatcggcggatatcgt

SEQ ID NO: 11 - DNA, 23 bp, Zea mays
  source 1..23: mol_type = genomic DNA
ccgagctcgaccacgccgccgac

SEQ ID NO: 12 - DNA, 24 bp, synthetic construct
  misc_feature 1..24: note = oligonucleotide C1-1F with sticky end
  source 1..24: mol_type = other DNA
agcagtcggcggcgtggtcgagct

SEQ ID NO: 13 - DNA, 24 bp, synthetic construct
  misc_feature 1..24: note = oligonucleotide C1-2F with sticky end
  source 1..24: mol_type = other DNA
ggcggtcggcggcgtggtcgagct

SEQ ID NO: 14 - DNA, 24 bp, synthetic construct
  misc_feature 1..24: note = oligonucleotide C1R with sticky end
  source 1..24: mol_type = other DNA
aaacagctcgaccacgccgccgac

SEQ ID NO: 15 - DNA, 21 bp, synthetic construct
  misc_feature 1..21: note = Forward Primer ZmIPK-1F
  source 1..21: mol_type = other DNA
tcgcagcccctggcagagcaa

SEQ ID NO: 16 - DNA, 26 bp, synthetic construct
  misc_feature 1..26: note = Reverse Primer ZmIPK-1R
  source 1..26: mol_type = other DNA
gagacctgggagaaggagacggatcc

SEQ ID NO: 17 - protein, 18 aa, synthetic construct
  REGION 1..18: note = solid powder CPPs (cell-penetrating peptides)
RKKRRQRRRRKKRRQRRR

SEQ ID NO: 18 - DNA, 22 bp, synthetic construct
  misc_feature 1..22: note = Forward Primer ZmU3-F
  source 1..22: mol_type = other DNA
ctgccaagatcaacagcaacca

SEQ ID NO: 19 - DNA, 22 bp, synthetic construct
  misc_feature 1..22: note = Forward Primer Cas9-1F
  source 1..22: mol_type = other DNA
cttcccaagcattccctcctgt

SEQ ID NO: 20 - DNA, 22 bp, synthetic construct
  misc_feature 1..22: note = Reverse Primer Cas9-1R
  source 1..22: mol_type = other DNA
cttatgccgtcccatgaccttc

SEQ ID NO: 21 - DNA, 25 bp, synthetic construct
  misc_feature 1..25: note = Forward Primer pBUE411-1F
  source 1..25: mol_type = other DNA
gacaggcgtcttctactggtgctac

SEQ ID NO: 22 - DNA, 22 bp, synthetic construct
  misc_feature 1..22: note = Forward Primer CAS9-2F
  source 1..22: mol_type = other DNA
ctccctaagcactcgctcctgt

SEQ ID NO: 23 - DNA, 22 bp, synthetic construct
  misc_feature 1..22: note = Reverse Primer CAS9-2R
  source 1..22: mol_type = other DNA
ttctgcgtggtctgattctccc

SEQ ID NO: 24 - DNA, 23 bp, Arabidopsis thaliana
  source 1..23: mol_type = genomic DNA
ccgacgatatccgccgatttcac

SEQ ID NO: 25 - DNA, 24 bp, synthetic construct
  misc_feature 1..24: note = Forward Primer C2F
  source 1..24: mol_type = other DNA
attggtgaaatcggcggatatcgt

SEQ ID NO: 26 - DNA, 24 bp, synthetic construct
  misc_feature 1..24: note = Reverse Primer C2R
  source 1..24: mol_type = other DNA
aaacacgatatccgccgatttcac

SEQ ID NO: 27 - DNA, 20 bp, synthetic construct
  misc_feature 1..20: note = Forward Primer PTPA-F
  source 1..20: mol_type = other DNA
gatgctccagccaccatatc

SEQ ID NO: 28 - DNA, 24 bp, synthetic construct
  misc_feature 1..24: note = Reverse Primer PTPA-R
  source 1..24: mol_type = other DNA
cagttcggtacaccacttatatca

SEQ ID NO: 29 - DNA, 25 bp, synthetic construct
  misc_feature 1..25: note = Forward Primer pHSN401-1F
  source 1..25: mol_type = other DNA
tgtcccaggattagaatgattaggc

SEQ ID NO: 30 - DNA, 55 bp, Zea mays
  source 1..55: mol_type = genomic DNA
ccatgctccaggtcgtctccgagctcgaccacgccgccgaccaggacagcacttt

SEQ ID NO: 31 - DNA, 54 bp, synthetic construct
  misc_feature 1..54: note = mutant ZmIPK target
  source 1..54: mol_type = other DNA
ccatgctccaggtcgtctccgagccgaccacgccgccgaccaggacagcacttt

SEQ ID NO: 32 - DNA, 56 bp, synthetic construct
  misc_feature 1..56: note = mutant ZmIPK target
  source 1..56: mol_type = other DNA
ccatgctccaggtcgtctccgagcatcgaccacgccgccgaccaggacagcacttt

SEQ ID NO: 33 - DNA, 47 bp, synthetic construct
  misc_feature 1..47: note = mutant ZmIPK target
  source 1..47: mol_type = other DNA
ccatgctccaggtcgtctccgcacgccgccgaccaggacagcacttt

SEQ ID NO: 34 - DNA, 45 bp, synthetic construct
  misc_feature 1..45: note = mutant ZmIPK target
  source 1..45: mol_type = other DNA
ccatgctccaggtcgtctccgagccgccgaccaggacagcacttt

SEQ ID NO: 35 - DNA, 50 bp, synthetic construct
  misc_feature 1..50: note = mutant ZmIPK target
  source 1..50: mol_type = other DNA
ccatgctccaggtcgtctccgagccacgccgccgaccaggacagcacttt

SEQ ID NO: 36 - DNA, 49 bp, synthetic construct
  misc_feature 1..49: note = mutant ZmIPK target
  source 1..49: mol_type = other DNA
ccatgctccaggtcgtctccgaccacgccgccgaccaggacagcacttt

SEQ ID NO: 37 - DNA, 53 bp, synthetic construct
  misc_feature 1..53: note = mutant ZmIPK target
  source 1..53: mol_type = other DNA
ccatgctccaggtcgtctccgagcgaccacgccgccgaccaggacagcacttt

SEQ ID NO: 38 - DNA, 56 bp, synthetic construct
  misc_feature 1..56: note = mutant ZmIPK target
  source 1..56: mol_type = other DNA
ccatgctccaggtcgtctccgagcttcgaccacgccgccgaccaggacagcacttt

SEQ ID NO: 39 - DNA, 48 bp, synthetic construct
  misc_feature 1..48: note = mutant ZmIPK target
  source 1..48: mol_type = other DNA
ccatgctccaggtcgtctccgacacgccgccgaccaggacagcacttt

SEQ ID NO: 40 - DNA, 44 bp, synthetic construct
  misc_feature 1..44: note = mutant ZmIPK target
  source 1..44: mol_type = other DNA
ccatgctccaggtcgtctccgagcgccgaccaggacagcacttt

SEQ ID NO: 41 - DNA, 46 bp, synthetic construct
  misc_feature 1..46: note = mutant ZmIPK target
  source 1..46: mol_type = other DNA
ccatgctccaggtcgtctccgagcccgccgaccaggacagcacttt

SEQ ID NO: 42 - DNA, 53 bp, synthetic construct; identical to SEQ ID NO: 37
  misc_feature 1..53: note = mutant ZmIPK target
  source 1..53: mol_type = other DNA

SEQ ID NO: 43 - DNA, 70 bp, Arabidopsis thaliana
  source 1..70: mol_type = genomic DNA
ctatcatttccaatctcccgtcaaacgaatccactctcccgacgatatccgccgatttcacgaatccgct

SEQ ID NO: 44 - DNA, 21 bp, synthetic construct
  misc_feature 1..21: note = mutant AtPTPA target
  source 1..21: mol_type = other DNA
ctatcatttcacgaatccgct

SEQ ID NO: 45 - DNA, 71 bp, synthetic construct
  misc_feature 1..71: note = mutant AtPTPA target
  source 1..71: mol_type = other DNA
ctatcatttccaatctcccgtcaaacgaatccactctcccgacgtatatccgccgatttcacgaatccgct

SEQ ID NO: 46 - DNA, 21 bp, synthetic construct
  misc_feature 1..21: note = mutant AtPTPA target
  source 1..21: mol_type = other DNA
ctatcatttcacgaatccgct

SEQ ID NO: 47 - DNA, 71 bp, synthetic construct; identical to SEQ ID NO: 45
  misc_feature 1..71: note = mutant AtPTPA target
  source 1..71: mol_type = other DNA

SEQ ID NO: 48 - DNA, 69 bp, synthetic construct
  misc_feature 1..69: note = mutant AtPTPA target
  source 1..69: mol_type = other DNA
ctatcatttccaatctcccgtcaaacgaatccactctcccgacatatccgccgatttcacgaatccgct

SEQ ID NO: 49 - DNA, 63 bp, synthetic construct
  misc_feature 1..63: note = mutant AtPTPA target
  source 1..63: mol_type = other DNA
ctatcatttccaatctcccgtcaaacgaatccactctcccgacgacgatttcacgaatccgct

SEQ ID NO: 50 - DNA, 60 bp, synthetic construct
  misc_feature 1..60: note = mutant AtPTPA target
  source 1..60: mol_type = other DNA
ctatcatttccaatctcccgtcaaacgaatccactctcccgacgatttcacgaatccgct

SEQ ID NO: 51 - DNA, 38 bp, synthetic construct
  misc_feature 1..38: note = mutant AtPTPA target
  source 1..38: mol_type = other DNA
ctatcatttccaatatccgccgatttcacgaatccgct